European Patent Application EP 4 410 833 A2, published August 7, 2024. Title: COMPOSITIONS AND METHODS FOR TREATING FATTY TISSUE BUILDUP. Applicant: MHS Care - Innovation LLC. The sequence listing filed with the application follows.

SEQUENCE LISTING (55 sequences)

SEQ ID NO: 1 - protein, 42 aa, Homo sapiens
YAEGTFISDYSIAMDKIHQQDFVNWLLAQKGKKNDWKHNITQ

SEQ ID NO: 2 - protein, 42 aa, Mus musculus
YAEGTFISDYSIAMDKIRQQDFVNWLLAQRGKKSDWKHNITQ

SEQ ID NO: 3 - protein, 42 aa, Rattus norvegicus
YAEGTFISDYSIAMDKIRQQDFVNWLLAQKGKKNDWKHNLTQ

SEQ ID NO: 4 - protein, 42 aa, Sus scrofa
YAEGTFISDYSIAMDKIRQQDFVNWLLAQKGKKSDWKHNITQ

SEQ ID NO: 5 - protein, 18 aa, synthetic construct
  REGION 1..18: note = artificial screening peptide
YAEGTFISDYSIAMDKIC

SEQ ID NO: 6 - protein, 18 aa, synthetic construct
  REGION 1..18: note = artificial screening peptide
CLLAQRGKKSDWKHNITQ

SEQ ID NO: 7 - protein, 109 aa, Mus musculus
DIQLTQSPAIMAASLGQKVTMTCSASSSVSSSYLHWYQQKSGASPKSLIHRTSNLASGVPARFSGSGSGTSYSLTISSVEAEDDATYYCLQWSGFPFTFGSGTKLEIKR

SEQ ID NO: 8 - DNA, 327 bp, synthetic construct
  misc_feature 1..327: note = artificial
  source 1..327: mol_type = other DNA
gacattcagctgacccagtctccagcaataatggctgcctctctggggcagaaggtcaccatgacctgcagtgccagctcaagtgtaagttccagttacttgcactggtaccagcagaagtcaggcgcttcccccaaatccttgattcataggacatccaacctggcttctggagtcccagctcgcttcagtggcagtgggtctgggacctcttactctctcacaatcagcagcgtggaggctgaagatgatgcaacttattactgcctgcagtggagtggtttcccattcacgttcggctcggggaccaagctggagatcaaacgt

SEQ ID NO: 9 - protein, 12 aa, Mus musculus
SASSSVSSSYLH

SEQ ID NO: 10 - protein, 9 aa, Mus musculus
LQWSGFPFT

SEQ ID NO: 11 - protein, 117 aa, Mus musculus
QVQLQESGAALVRSGASVKLSCTASGFNIKDYYFHWVKQRPDQGLEWIGWIDPENGDTEYAPNFQVKATMTADTYSNTAYLHLSSLTSEDTAVYYCNSYGNNYFDYWGQGTTVTVSS

SEQ ID NO: 12 - DNA, 351 bp, synthetic construct
  misc_feature 1..351: note = artificial
  source 1..351: mol_type = other DNA
caggtccagctgcaggagtctggggcagcgcttgtgaggtcaggggcctcagtcaaattgtcctgcacagcttctggcttcaacattaaagactactattttcactgggtgaagcagaggcctgaccagggcctggagtggattggatggattgatcctgagaatggtgatactgaatatgccccgaacttccaggtcaaggccactatgactgcagacacatattccaacacagcctacctgcatctcagcagcctgacatctgaggacactgccgtctattactgtaattcctacggtaataactactttgactactggggccaagggaccacggtcaccgtctcctca

SEQ ID NO: 13 - protein, 10 aa, Mus musculus
GFNIKDYYFH

SEQ ID NO: 14 - protein, 7 aa, Mus musculus
APNFQVK

SEQ ID NO: 15 - protein, 10 aa, Mus musculus
NSYGNNYFDY

SEQ ID NO: 16 - protein, 111 aa, Mus musculus
DIQLTQSPSTMAASPGEKITITCSASSSISSNSLHWYQQKPGFSPKLLIYRTSNLASGVPGRFSGSGSGTSYSLTIGTMETEDVATYYCQQGSSFPRMLTFGTGTKLEIKR

SEQ ID NO: 17 - protein, 111 aa, synthetic construct
  REGION 1..111: note = humanized
DIQMTQSPSSVSASVGDRVTITCRASSSISSNSLHWYQQKPGKAPKLLIYRTSSLQSGVPSRFSGSGSGTDYTLTISSLQPEDFATYYCQQGSSFPRMLTFGQGTKLEIKR

SEQ ID NO: 18 - protein, 111 aa, synthetic construct
  REGION 1..111: note = humanized
DIQLTQSPSSVSASVGDRVTITCRASSSISSNSLHWYQQKPGKAPKLLIYRTSNLQSGVPSRFSGSGSGTDYTLTISSLQPEDFATYYCQQGSSFPRMLTFGQGTKLEIKR

SEQ ID NO: 19 - protein, 111 aa, synthetic construct
  REGION 1..111: note = humanized
DIQMTQSPGTLSLSPGERATLSCRASSSISSNSLHWYQQKPGQAPRLLIYRTSNRATGIPARFSGSGSGTDYTLTISSLEPEDFAVYYCQQGSSFPRMLTFGGGTKVEIKR

SEQ ID NO: 20 - protein, 12 aa, synthetic construct
  REGION 1..12: note = humanized
RASSSISSNSLH

SEQ ID NO: 21 - protein, 7 aa, synthetic construct
  REGION 1..7: note = humanized
RTSNLQS

SEQ ID NO: 22 - protein, 11 aa, synthetic construct
  REGION 1..11: note = HUMANIZED
QQGSSFPRMLT

SEQ ID NO: 23 - protein, 7 aa, synthetic construct
  REGION 1..7: note = HUMANIZED
RTSSLQS

SEQ ID NO: 24 - protein, 7 aa, synthetic construct
  REGION 1..7: note = HUMANIZED
RTSNRAT

SEQ ID NO: 25 - protein, 12 aa, synthetic construct
  REGION 1..12: note = HUMANIZED
SASSSISSNSLH

SEQ ID NO: 26 - protein, 7 aa, Mus musculus
RTSNLAS

SEQ ID NO: 27 - protein, 117 aa, Mus musculus
QVQLQESGAELVRSGASVKLSCTASGFNIRDYYLHWIKQRPEQGLEWIGWIDPENGDTEYAPKFQDKATVTADTSSNTAYLQLNSLTSEDTAVYYCNVYGIYFMDYWGQGTTVTVSS

SEQ ID NO: 28 - protein, 117 aa, synthetic construct
  REGION 1..117: note = HUMANIZED
QVQLVQSGAEVKKPGATVKISCKVSGFNIRDYYLHWVQQAPGKGLEWMGWIDPENGDTEYAPKFQGRVTITADTSTDTAYMELSSLRSEDTAVYYCNVYGIYFMDYWGQGTMVTVSS

SEQ ID NO: 29 - protein, 117 aa, synthetic construct
  REGION 1..117: note = HUMANIZED
QVQLVQSGAEVKKPGATVKISCKASGFNIRDYYLHWVQQAPGKGLEWMGWIDPENGDTEYAPKFQGRVTITADTSTNTAYMELSSLRSEDTAVYYCNVYGIYFMDYWGQGTMVTVSS

SEQ ID NO: 30 - protein, 117 aa, synthetic construct
  REGION 1..117: note = HUMANIZED
QVQLQESGAEVKKPGASVKVSCKASGFNIRDYYLHWVRQAPGQGLEWMGWIDPENGDTEYAPKFQGRVTTTADTSISTAYMELSRLRSDDTAVYYCNVYGIYFMDYWGQGTLVTVSS

SEQ ID NO: 31 - protein, 10 aa, Mus musculus
GFNIRDYYLH

SEQ ID NO: 32 - protein, 7 aa, synthetic construct
  REGION 1..7: note = HUMANIZED
APKFQGR

SEQ ID NO: 33 - protein, 10 aa, Mus musculus
NVYGIYFMDY

SEQ ID NO: 34 - protein, 7 aa, Mus musculus
APKFQDK

SEQ ID NO: 35 - DNA, 333 bp, synthetic construct
  misc_feature 1..333: note = ARTIFICIAL
  source 1..333: mol_type = other DNA
gacattcagctgacccagtctccatccaccatggctgcatctcccggggagaagatcactatcacctgcagtgccagctcaagtataagttccaattccttgcattggtatcagcagaagccaggattctcccctaaactcttgatttataggacatccaatctggcttctggagtcccaggtcgcttcagtggcagtgggtctgggacctcttactctctcacaattggcaccatggagactgaagatgttgccacttactactgccagcagggtagtagttttccacgcatgctcacgttcggtactgggaccaagctggagatcaaacgt

SEQ ID NO: 36 - DNA, 333 bp, synthetic construct
  misc_feature 1..333: note = ARTIFICIAL
  source 1..333: mol_type = other DNA
gacatccagatgacccagtccccctcctccgtgtctgcttctgtgggcgacagagtgacaattacctgccgggcctcctcctccatctcctccaattccctgcactggtatcagcagaagcccggcaaggcccccaagctgctgatctaccggacctccagcctgcagtccggcgtgccctctagattctccggctctggctctggcaccgactataccctgaccatctccagcctgcagcccgaggacttcgccacctactactgtcagcagggctcctccttcccccggatgctgacatttggccagggcaccaagctggaaatcaagcgg

SEQ ID NO: 37 - DNA, 333 bp, synthetic construct
  misc_feature 1..333: note = ARTIFICIAL
  source 1..333: mol_type = other DNA
gacatccagctgacccagtccccctcctccgtgtctgcttctgtgggcgacagagtgacaattacctgccgggcctcctcctccatctcctccaattccctgcactggtatcagcagaagcccggcaaggcccccaagctgctgatctaccggacctccaacctgcagtccggcgtgccctctagattctccggctctggctctggcaccgactataccctgaccatctccagcctgcagcccgaggacttcgccacctactactgtcagcagggctcctccttcccccggatgctgacatttggccagggcaccaagctggaaatcaagcgg

SEQ ID NO: 38 - DNA, 333 bp, synthetic construct
  misc_feature 1..333: note = ARTIFICIAL
  source 1..333: mol_type = other DNA
gacatccagatgacccagagccctggcaccctgtctctgtctcccggcgagagagctaccctgtcctgcagagcctcctcctccatctcctccaattccctgcactggtatcagcagaagcccggccaggcccccagactgctgatctaccggacctccaatcgggccaccggcatccctgccagattctccggctctggctctggcaccgactataccctgaccatctccagcctggaacccgaggacttcgccgtgtactactgtcagcagggctcctccttcccccggatgctgacatttggcggaggcaccaaggtggaaatcaagcgg

SEQ ID NO: 39 - DNA, 351 bp, synthetic construct
  misc_feature 1..351: note = ARTIFICIAL
  source 1..351: mol_type = other DNA
caggtccagctgcaggagtctggggcagagcttgtgaggtcaggggcctcagtcaagttgtcctgcacagcttctggcttcaacattagagactactatttgcactggataaaacagaggcctgaacagggcctggagtggattggatggattgatcctgagaatggtgatactgaatatgccccgaagttccaggacaaggccactgtgactgcagacacatcctccaacacagcctacctgcagctcaacagcctgacatctgaggacactgccgtctattactgtaatgtatatggcatctattttatggactattggggccaagggaccacggtcaccgtctcctca

SEQ ID NO: 40 - DNA, 351 bp, synthetic construct
  misc_feature 1..351: note = ARTIFICIAL
  source 1..351: mol_type = other DNA
caggtgcagctggtgcagtctggcgccgaagtgaagaaacctggcgctaccgtgaagatctcctgcaaggtgtccggcttcaacatccgggactactacctgcactgggtgcagcaggcccctggcaagggactggaatggatgggctggatcgaccccgagaacggcgataccgagtacgcccctaagttccagggcagagtgaccatcaccgccgacacctctaccgacaccgcctacatggaactgtcctccctgcggagcgaggacaccgccgtgtactactgcaacgtgtacggcatctacttcatggactactggggccagggcacaatggtcaccgtgtcctct

SEQ ID NO: 41 - DNA, 351 bp, synthetic construct
  misc_feature 1..351: note = ARTIFICIAL
  source 1..351: mol_type = other DNA
caggtgcagctggtgcagtctggcgccgaagtgaagaaacctggcgctaccgtgaagatctcctgcaaggcctccggcttcaacatccgggactactacctgcactgggtgcagcaggcccctggcaagggactggaatggatgggctggatcgaccccgagaacggcgataccgagtacgcccctaagttccagggcagagtgaccatcaccgccgacacctctaccaacaccgcctacatggaactgtcctccctgcggagcgaggacaccgccgtgtactactgcaacgtgtacggcatctacttcatggactactggggccagggcacaatggtcaccgtgtcctct

SEQ ID NO: 42 - DNA, 351 bp, synthetic construct
  misc_feature 1..351: note = artificial
  source 1..351: mol_type = other DNA
caggtgcagctgcaggaatctggcgccgaagtgaagaaacctggcgcctccgtgaaggtgtcctgcaaggcctccggcttcaacatccgggactactacctgcactgggtgcgacaggctccaggccagggactggaatggatgggctggatcgaccccgagaacggcgataccgagtacgcccctaagttccagggcagagtgaccaccaccgccgacacctctatctccaccgcctacatggaactgtcccggctgagatccgacgacaccgccgtgtactactgcaacgtgtacggcatctacttcatggactactggggccagggcacactcgtcaccgtgtcctct

SEQ ID NO: 43 - protein, 46 aa, synthetic construct
  REGION 1..46: note = primer
CAGTCGAAGCTTTGAGGAGACGGTGACCGTGGTCCCTTGGCCCCAG

SEQ ID NO: 44 - protein, 34 aa, synthetic construct
  REGION 1..34: note = primer
CAACTAGGATCCAGGTSMARCTGCAGSAGTCWGG

SEQ ID NO: 45 - protein, 6 aa, synthetic construct
  REGION 1..6: note = primer
AAGCTT

SEQ ID NO: 46 - protein, 6 aa, synthetic construct
  REGION 1..6: note = primer
GGATCC

SEQ ID NO: 47 - protein, 34 aa, synthetic construct
  REGION 1..34: note = primer
CAGTCGAAGCTTGTTAGATCTCCAGCTTGGTCCC

SEQ ID NO: 48 - DNA, 36 bp, synthetic construct
  misc_feature 1..36: note = primer
  source 1..36: mol_type = other DNA
caactaggatccgacattcagctgacccagtctcca

SEQ ID NO: 49 - DNA, 30 bp, synthetic construct
  misc_feature 1..30: note = primer
  source 1..30: mol_type = other DNA
tcacgaattctcaggtccagctgcaggagt

SEQ ID NO: 50 - DNA, 29 bp, synthetic construct
  misc_feature 1..29: note = primer
  source 1..29: mol_type = other DNA
ttggtgctagctgaggagacggtgaccgt

SEQ ID NO: 51-52 - skipped (2 entries)

SEQ ID NO: 53 - DNA, 34 bp, synthetic construct
  misc_feature 1..34: note = primer
  source 1..34: mol_type = other DNA
agccaccgtacgtttgatctccagcttggtccca

SEQ ID NO: 54 - skipped

SEQ ID NO: 55 - protein, 30 aa, synthetic construct
  REGION 1..30: note = primer
GTCACGAATTCAGACATTCAGCTGACCCAG